European Patent Application EP 4 235 677 A2, published August 30, 2023. Title: PROCESSES AND SYSTEMS FOR NUCLEIC ACID SEQUENCE ASSEMBLY. Applicant: 10X Genomics, Inc. The sequence listing filed with the application follows.

SEQUENCE LISTING (1 sequence)

SEQ ID NO: 1 - DNA, 10 bp, synthetic construct
  misc_feature 1..10: note = Sequence of Figure 10
  source 1..10: mol_type = other DNA
gatccatctt